European Patent Specification EP 3 592 351 B1, published May 10, 2023. Title: Use of serine protease inhibitors, in particular of serpinB3. Applicant: Università degli studi di Padova. The sequence listing filed with the application follows.

SEQUENCE LISTING (4 sequences)

SEQ ID NO: 1 - DNA, 20 bp, Artificial Sequence
  source 1..20: /mol_type="unassigned DNA" /note="primer senso per Serpin B3" /organism="Artificial Sequence"
gcaaatgctccagaagaaag

SEQ ID NO: 2 - DNA, 21 bp, Artificial Sequence
  source 1..21: /mol_type="unassigned DNA" /note="primer antisenso Serpin B3" /organism="Artificial Sequence"
cgaggcaaaatgaaaaagatg

SEQ ID NO: 3 - DNA, 25 bp, Artificial Sequence
  source 1..25: /mol_type="unassigned DNA" /note="primer senso HPRT1" /organism="Artificial Sequence"
tcaggcagtataatccaaagatggt

SEQ ID NO: 4 - DNA, 20 bp, Artificial Sequence
  source 1..20: /mol_type="unassigned DNA" /note="primer antisenso HPRT1" /organism="Artificial Sequence"
cttcgtggggtccttttcac